European Patent Application EP 4 524 821 A2, published March 19, 2025. Title: High-Capacity Storage of Digital Information in DNA. Applicant: European Molecular Biology Laboratory. Application EP PCT/EP2013/061300, filed May 13, 2013. The sequence listing filed with the application follows.

SEQUENCE LISTING (4 sequences)

SEQ ID NO: 1 - DNA, 33 bp, synthetic construct
  misc_feature 1..33: note = 5' Sequencing Adapter
  source 1..33: mol_type = other DNA
acactctttccctacacgacgctcttccgatct

SEQ ID NO: 2 - DNA, 33 bp, synthetic construct
  misc_feature 1..33: note = 3' Sequencing Adapter
  source 1..33: mol_type = other DNA
agatcggaagagcggttcagcaggaatgccgag

SEQ ID NO: 3 - DNA, 20 bp, synthetic construct
  misc_feature 1..20: note = 20bp motif with self reverse complementary pattern
  source 1..20: mol_type = other DNA
gagcatctgcagatgctcat

SEQ ID NO: 4 - DNA, 75 bp, synthetic construct
  misc_feature 1..75: note = information encoding DNA
  source 1..75: mol_type = other DNA
tagatgtgtacagactacgcgcagcgagatcgactcgcagtgctgagtgacagactagtcacgtcgcagcgctag